European Patent Application EP 4 484 958 A1, published January 1, 2025. Title: Targeted proteomics for autophagy detection. Applicant: University of Fribourg. The sequence listing filed with the application follows.

SEQUENCE LISTING (97 sequences)

SEQ ID NO: 1 - protein, 15 aa, Homo sapiens
TVGVAFNQETGHWER

SEQ ID NO: 2 - protein, 15 aa, Homo sapiens
WLPEPGLGLAYGTNK

SEQ ID NO: 3 - protein, 10 aa, Homo sapiens
TIQGLIDFIK

SEQ ID NO: 4 - protein, 13 aa, Homo sapiens
ASPHDVLETIFVR

SEQ ID NO: 5 - protein, 21 aa, Homo sapiens
EGGVPLAPNQPVHGTQADQER

SEQ ID NO: 6 - protein, 16 aa, Homo sapiens
SSSSPTGSDWFNLAIK

SEQ ID NO: 7 - protein, 11 aa, Homo sapiens
DLADALLDTER

SEQ ID NO: 8 - protein, 11 aa, Homo sapiens
DLLWLPIEQYR

SEQ ID NO: 9 - protein, 14 aa, Homo sapiens
FTSEVPIWLDYHGK

SEQ ID NO: 10 - protein, 13 aa, Homo sapiens
ALEVAEYLTPVLK

SEQ ID NO: 11 - protein, 15 aa, Homo sapiens
FVQAVIPTIEYDYTR

SEQ ID NO: 12 - protein, 13 aa, Homo sapiens
TDAGGEDAILQTR

SEQ ID NO: 13 - protein, 15 aa, Homo sapiens
LGINQINPVYVDAFK

SEQ ID NO: 14 - protein, 8 aa, Homo sapiens
LLSDISAR

SEQ ID NO: 15 - protein, 16 aa, Homo sapiens
SIGEWFGPNTVAQVLK

SEQ ID NO: 16 - protein, 11 aa, Homo sapiens
EAEPYYLLLPR

SEQ ID NO: 17 - protein, 15 aa, Homo sapiens
IPTCFTLYQDEITER

SEQ ID NO: 18 - protein, 10 aa, Homo sapiens
VSYLTLVTDK

SEQ ID NO: 19 - protein, 11 aa, Homo sapiens
DVAHSIIFEVK

SEQ ID NO: 20 - protein, 14 aa, Homo sapiens
GYYYNGDSAGLPAR

SEQ ID NO: 21 - protein, 9 aa, Homo sapiens
ALEIIDFFR

SEQ ID NO: 22 - protein, 24 aa, Homo sapiens
LEASYSDSPPGEEDLLVHVAEGSK

SEQ ID NO: 23 - protein, 14 aa, unidentified
SFSPLQPGQAPTGR

SEQ ID NO: 24 - protein, 11 aa, Homo sapiens
AELLQGGDLLR

SEQ ID NO: 25 - protein, 10 aa, Homo sapiens
TILDANEEFK

SEQ ID NO: 26 - protein, 12 aa, Homo sapiens
ASETDTHSIGEK

SEQ ID NO: 27 - protein, 11 aa, Homo sapiens
ILLDAQHESGR

SEQ ID NO: 28 - protein, 15 aa, Homo sapiens
DHSSQSEEEVVEGEK

SEQ ID NO: 29 - protein, 15 aa, Homo sapiens
ILLDAQHESGQSSSR

SEQ ID NO: 30 - protein, 11 aa, Homo sapiens
DYWETELLQLK

SEQ ID NO: 31 - protein, 13 aa, Homo sapiens
ENDHLFLSLTEQR

SEQ ID NO: 32 - protein, 7 aa, Homo sapiens
LEQELLK

SEQ ID NO: 33 - protein, 12 aa, Homo sapiens
FFLNGVFIHDQK

SEQ ID NO: 34 - protein, 14 aa, Homo sapiens
GELQQLSGSQLHGK

SEQ ID NO: 35 - protein, 24 aa, Homo sapiens
IPEDSIYIGTASDDSDIVTLEPPK

SEQ ID NO: 36 - protein, 12 aa, Homo sapiens
LDFGIGEYINQK

SEQ ID NO: 37 - protein, 18 aa, Homo sapiens
SLSESWEVINSKPDERPR

SEQ ID NO: 38 - protein, 15 aa, Homo sapiens
ADFVLAANSYDLAIK

SEQ ID NO: 39 - protein, 16 aa, Homo sapiens
VLAQQGEYSEAIPILR

SEQ ID NO: 40 - protein, 8 aa, Homo sapiens
EDHPFEYR

SEQ ID NO: 41 - protein, 7 aa, Homo sapiens
IQLPSEK

SEQ ID NO: 42 - protein, 11 aa, Homo sapiens
VSGSQIVDIDK

SEQ ID NO: 43 - protein, 11 aa, Homo sapiens
GALSVAASAYK

SEQ ID NO: 44 - protein, 14 aa, Homo sapiens
IHLWNSIHGLQSPK

SEQ ID NO: 45 - protein, 11 aa, Homo sapiens
VSFDLNTIQIK

SEQ ID NO: 46 - protein, 11 aa, Homo sapiens
DLELAIGGVLR

SEQ ID NO: 47 - protein, 11 aa, Homo sapiens
DFFGLDTNSAK

SEQ ID NO: 48 - protein, 12 aa, Homo sapiens
DYHNYQTLFEPR

SEQ ID NO: 49 - protein, 13 aa, Homo sapiens
ADLLGIVSELQLK

SEQ ID NO: 50 - protein, 15 aa, Homo sapiens
LNSSGSSEDSFVEIR

SEQ ID NO: 51 - protein, 13 aa, Homo sapiens
TSDSDQQAYLVQR

SEQ ID NO: 52 - protein, 17 aa, Homo sapiens
IGGVQQDTILAEGLHFR

SEQ ID NO: 53 - protein, 12 aa, Homo sapiens
IVQAEGEAEAAK

SEQ ID NO: 54 - protein, 13 aa, Homo sapiens
LLLGAGAVAYGVR

SEQ ID NO: 55 - protein, 15 aa, Homo sapiens
VSDGENVIISHFNSK

SEQ ID NO: 56 - protein, 16 aa, Homo sapiens
YVDGGISDNLPLYELK

SEQ ID NO: 57 - protein, 11 aa, Homo sapiens
ELAQGFLANQK

SEQ ID NO: 58 - protein, 11 aa, Homo sapiens
SLLEQETENLR

SEQ ID NO: 59 - protein, 9 aa, Homo sapiens
FSPGDFWGR

SEQ ID NO: 60 - protein, 10 aa, Homo sapiens
HINWEELLAR

SEQ ID NO: 61 - protein, 18 aa, Homo sapiens
LGAGPGDAGEVQAHPFFR

SEQ ID NO: 62 - protein, 19 aa, Homo sapiens
TTPPVEVLHENESGGSEIK

SEQ ID NO: 63 - protein, 13 aa, Homo sapiens
VEGIYTYSLSPSK

SEQ ID NO: 64 - protein, 15 aa, Homo sapiens
EAALYPHLPPEADPR

SEQ ID NO: 65 - protein, 18 aa, Homo sapiens
LAFPSPFGHLSEGFSHSR

SEQ ID NO: 66 - protein, 14 aa, Homo sapiens
LTPVSPESSSTEEK

SEQ ID NO: 67 - protein, 15 aa, Homo sapiens
NYDIGAALDTIQYSK

SEQ ID NO: 68 - protein, 9 aa, Homo sapiens
VAALFPALR

SEQ ID NO: 69 - protein, 23 aa, Homo sapiens
EHVPSGQFPDTEAPATSETSNSR

SEQ ID NO: 70 - protein, 11 aa, Homo sapiens
FVLVENGGVTR

SEQ ID NO: 71 - protein, 14 aa, Homo sapiens
HSSWGDVGVGGSLK

SEQ ID NO: 72 - protein, 14 aa, Homo sapiens
AHQLEEDIVSVTHK

SEQ ID NO: 73 - protein, 14 aa, Homo sapiens
LSDQSANNNNVFTK

SEQ ID NO: 74 - protein, 7 aa, Homo sapiens
ANDLDVR

SEQ ID NO: 75 - protein, 10 aa, Homo sp.
EYLSETYGNK

SEQ ID NO: 76 - protein, 13 aa, Homo sapiens
FAAHISPAQGSPK

SEQ ID NO: 77 - protein, 23 aa, Homo sapiens
FAAHISPAQGSPKPPPAASPGVR

SEQ ID NO: 78 - protein, 19 aa, Homo sapiens
IYDPGGSVPSGEASAAFER

SEQ ID NO: 79 - protein, 13 aa, Homo sapiens
LQAQVTLSNAQLK

SEQ ID NO: 80 - protein, 14 aa, Homo sapiens
GPVYIGELPQDFLR

SEQ ID NO: 81 - protein, 13 aa, Homo sapiens
IAWTHITIPESLR

SEQ ID NO: 82 - protein, 16 aa, Homo sapiens
LGYAVYETPTAHNGAK

SEQ ID NO: 83 - protein, 12 aa, Homo sapiens
APFQASSPQDLR

SEQ ID NO: 84 - protein, 7 aa, Homo sapiens
LPDFLQR

SEQ ID NO: 85 - protein, 8 aa, Homo sapiens
TLSEDTIR

SEQ ID NO: 86 - protein, 8 aa, Homo sapiens
TLVPTIPR

SEQ ID NO: 87 - protein, 13 aa, Homo sapiens
TPSSQNLLALLAR

SEQ ID NO: 88 - protein, 17 aa, Homo sapiens
VAELLSSGLQSAIDQIR

SEQ ID NO: 89 - protein, 8 aa, Homo sapiens
TLSEDTIR

SEQ ID NO: 90 - protein, 14 aa, Homo sapiens
AEAGGGWEGSASYK

SEQ ID NO: 91 - protein, 10 aa, Homo sapiens
QPVFGANYIK

SEQ ID NO: 92 - protein, 14 aa, Homo sapiens
DGFIFVNYSEGQTR

SEQ ID NO: 93 - protein, 16 aa, Homo sapiens
SEGVVPSPVSLVPEEK

SEQ ID NO: 94 - protein, 16 aa, Homo sapiens
EKPPEEPTTWTGYFGK

SEQ ID NO: 95 - protein, 9 aa, Homo sapiens
FFSLSSVDK

SEQ ID NO: 96 - protein, 10 aa, Homo sapiens
GTYVPSSPTR

SEQ ID NO: 97 - protein, 9 aa, Homo sapiens
VFSIPEGQK